European Patent Application EP 4 725 966 A1, published April 15, 2026. Title: 人表皮生长因子3的抗体、其制备方法及其应用. Applicant: 上海偌妥生物科技有限公司. Application CN. The sequence listing filed with the application follows.

SEQUENCE LISTING (37 sequences)

SEQ ID NO: 1 - protein, 112 aa, Mus musculus
DIVLTQSPASLAVSLGQRATISCRASESVDNYGIRLMHWYQQKSGQPPKLLIHRASNLESGIPARFSGSGSRTDFTLTINPVETDDVATYYCQQSNKDPFTFGSGTKLEIKR

SEQ ID NO: 2 - protein, 119 aa, Mus musculus
EVKLQESGPGLVKPSQSLSLTCSVTGYSITSGYYWNWIRQFPGNKLEWMGYISYDGSNNYNPSLKNRISITRDTSKNQFFLNLNSVTTEDTATYYCARVDWDGDAMDYWGQGTSVTVSS

SEQ ID NO: 3 - protein, 112 aa, Mus musculus
DIVLTQSPASLAVSLGQRATISCRASESVDNYGISLMHWYQQKPGQPPKLLIYRASNLESGIPARFSGSGSRTDFTLTINPVETDDVATYYCQQSNKDPPTFGAGTKLELKR

SEQ ID NO: 4 - protein, 119 aa, Mus musculus
EVKLQESGPGLVKPSQSLSLTCSVTGYSITSGYYWNWIRQFPGNKLEWMGYISYDGSNNYNPSLKNRISITRDTSKNQFFLKLNSVTTEDTATYYCARMDWDGDAMDYWGQGTSVTVSS

SEQ ID NO: 5 - protein, 108 aa, Mus musculus
DIQMTQSPASLSASVEETVTITCRASENIYSYLAWYQQKQGKSPQLLVYNAKTLAEGVPSRFSGSGSGTEFSLKINSLQPEDFGSYYCQNHYGTPYTFGGGTKLEIKQ

SEQ ID NO: 6 - protein, 122 aa, Mus musculus
EVQLVESGGGLVKPGGSLKLSCAASGFTFSSYVMSWVRQTPEKRLEWVATISDGDSSTYYPDNVKGRFTISRDNAKNNLFLQMSHLKSEDTAMYFCARDKGHGYDEGAFVYWGQGTLVTVSA

SEQ ID NO: 7 - protein, 112 aa, Mus musculus
DIVLTQSPASLAVSLGQRATISCRASESVDHYGSSFMHWYQQKPGQPPKLLIYRASNPESGIPARFSGSGSRTDFTLTINPVETDDVATYYCQQSNKDPPTFGGGTKLEIKR

SEQ ID NO: 8 - protein, 119 aa, Mus musculus
EVQLQESGPGLVKPSQSLSLTCSVTGYSITSGYYWNWIRQFPGNKLEWMGYISYDGSNNYNPSLKNRISITRDTSKNQFFLKLNSVTTEDTATYYCASYDYDGDWFAYWGQGTLVTVSA

SEQ ID NO: 9 - protein, 107 aa, Mus musculus
DIELTQSPALMSASPGEKVTMTCSASSSVSYMYWYQQKPRSSPKPWIYLTSNLASGVPARFSGSGSGTSYSLTISSMEAEDAATYYCQQWSRNPLTFGAGTKLELKR

SEQ ID NO: 10 - protein, 120 aa, Mus musculus
EVQLQQSGPDLVKPGTSVKMSCKASGYTFTDYYMHWVRQSHGKSLEWIGYINPNNGDAIYNQKFKGKATLTVNKSSTTAYMALRSLTSEDSAVYFCATYDYGGDFYFDVWGTGTTVTVSS

SEQ ID NO: 11 - protein, 120 aa, Mus musculus
EVQLQQSGPDLVKPGTSVKMSCKASGYTFTDYYMHWVRQSHGKSLEWIGYINPNNGDAIYNQKFKGKATLTVDKSSTTAYMALRSLTSEDSAVYFCATYDYGGDFYFDVWGTGTTVTVSS

SEQ ID NO: 12 - protein, 15 aa, Mus musculus
RASESVDNYGIRLMH

SEQ ID NO: 13 - protein, 7 aa, Mus musculus
RASNLES

SEQ ID NO: 14 - protein, 9 aa, Mus musculus
QQSNKDPFT

SEQ ID NO: 15 - protein, 9 aa, Mus musculus
SITSGYYWN

SEQ ID NO: 16 - protein, 11 aa, Mus musculus
MGYISYDGSNN

SEQ ID NO: 17 - protein, 12 aa, Mus musculus
ARVDWDGDAMDY

SEQ ID NO: 18 - protein, 15 aa, Mus musculus
RASESVDNYGISLMH

SEQ ID NO: 19 - protein, 9 aa, Mus musculus
QQSNKDPPT

SEQ ID NO: 20 - protein, 12 aa, Mus musculus
ARMDWDGDAMDY

SEQ ID NO: 21 - protein, 11 aa, Mus musculus
RASENIYSYLA

SEQ ID NO: 22 - protein, 7 aa, Mus musculus
NAKTLAE

SEQ ID NO: 23 - protein, 9 aa, Mus musculus
QNHYGTPYT

SEQ ID NO: 24 - protein, 8 aa, Mus musculus
TFSSYVMS

SEQ ID NO: 25 - protein, 12 aa, Mus musculus
VATISDGDSSTY

SEQ ID NO: 26 - protein, 15 aa, Mus musculus
ARDKGHGYDEGAFVY

SEQ ID NO: 27 - protein, 15 aa, Mus musculus
RASESVDHYGSSFMH

SEQ ID NO: 28 - protein, 7 aa, Mus musculus
RASNPES

SEQ ID NO: 29 - protein, 12 aa, Mus musculus
ASYDYDGDWFAY

SEQ ID NO: 30 - protein, 10 aa, Mus musculus
SASSSVSYMY

SEQ ID NO: 31 - protein, 7 aa, Mus musculus
LTSNLAS

SEQ ID NO: 32 - protein, 9 aa, Mus musculus
QQWSRNPLT

SEQ ID NO: 33 - protein, 8 aa, Mus musculus
TFTDYYMH

SEQ ID NO: 34 - protein, 12 aa, Mus musculus
IGYINPNNGDAI

SEQ ID NO: 35 - protein, 13 aa, Mus musculus
ATYDYGGDFYFDV

SEQ ID NO: 36 - protein, 108 aa, synthetic construct
DIQMTQSPSSLSASVGDRVTITCRASENIYSYLAWYQQKPGKAPKLLIYNAKTLAEGVPSRFSGSGSGTDFTLTISSLQPEDFATYYCQNHYGTPYTFGQGTKLEIKR

SEQ ID NO: 37 - protein, 122 aa, synthetic construct
QVQLVESGGGLVKPGGSLRLSCAASGFTFSSYVMSWVRQAPGKGLEWVATISDGDSSTYYADSVKGRFTISRDNAKNSLYLQMNSLRAEDTAVYYCARDKGHGYDEGAFVYWGQGTLVTVSS